European Patent Application EP 4 516 923 A1, published March 5, 2025. Title: DIGESTED DDIT4L PRODUCT AS DIAGNOSTIC MARKER FOR ALZHEIMER'S DISEASE. Applicant: PLASMARKER BIOTECHNOLOGY CO.,LTD. Application EP. The sequence listing filed with the application follows.

SEQUENCE LISTING (95 sequences)

SEQ ID NO: 1 - protein, 84 aa, Homo sapiens
MVATGSLSSKNPASISELLDCGYHPESLLSGECPRCPPFSPPKVGASGSIGWAGFRLPPLPLCRRCHKIHLRRLLSKFSNIFSP

SEQ ID NO: 2 - protein, 30 aa, synthetic construct
  REGION 1..30: note = Amino acids encoded by the first exon
MVATGSLSSKNPASISELLDCGYHPESLLS

SEQ ID NO: 3 - protein, 54 aa, synthetic construct
  REGION 1..54: note = Amino acids encoded by retained introns
GECPRCPPFSPPKVGASGSIGWAGFRLPPLPLCRRCHKIHLRRLLSKFSNIFSP

SEQ ID NO: 4 - protein, 27 aa, synthetic construct
  REGION 1..27: note = IR-1
GECPRCPPFSPPKVGASGSIGWAGFRL

SEQ ID NO: 5 - protein, 27 aa, synthetic construct
  REGION 1..27: note = IR-2
PPLPLCRRCHKIHLRRLLSKFSNIFSP

SEQ ID NO: 6 - DNA, 20 bp, synthetic construct
  misc_feature 1..20: note = forward primer
  source 1..20: mol_type = other DNA
tgctggactgtggctatcac

SEQ ID NO: 7 - DNA, 21 bp, synthetic construct
  misc_feature 1..21: note = reverse primer
  source 1..21: mol_type = other DNA
acaaggacctttgagcaacca

SEQ ID NO: 8 - DNA, 255 bp, synthetic construct
  misc_feature 1..255: note = DIR open reading frame
  source 1..255: mol_type = other DNA
atggttgcaactggcagtttgagcagcaagaacccggccagcatttcagaattgctggactgtggctatcacccagagagcctgctaagtggtgagtgtccccgctgtccacccttctcccctcccaaggtcggtgcctctggatctattgggtgggcgggctttcgacttcctcccctacctctatgtaggaggtgccacaaaatccatctgaggagactcctttccaaattttctaacatcttctctccatga

SEQ ID NO: 9 - DNA, 2346 bp, synthetic construct
  misc_feature 1..2346: note = Gelsolin open reading frame
  source 1..2346: mol_type = other DNA
atggctccgcaccgccccgcgcccgcgctgctttgcgcgctgtccctggcgctgtgcgcgctgtcgctgcccgtccgcgcggccactgcgtcgcggggggcgtcccaggcgggggcgccccaggggcgggtgcccgaggcgcggcccaacagcatggtggtggaacaccccgagttcctcaaggcagggaaggagcctggcctgcagatctggcgtgtggagaagttcgatctggtgcccgtgcccaccaacctttatggagacttcttcacgggcgacgcctacgtcatcctgaagacagtgcagctgaggaacggaaatctgcagtatgacctccactactggctgggcaatgagtgcagccaggatgagagcggggcggccgccatctttaccgtgcagctggatgactacctgaacggccgggccgtgcagcaccgtgaggtccagggcttcgagtcggccaccttcctaggctacttcaagtctggcctgaagtacaagaaaggaggtgtggcatcaggattcaagcacgtggtacccaacgaggtggtggtgcagagactcttccaggtcaaagggcggcgtgtggtccgtgccaccgaggtacctgtgtcctgggagagcttcaacaatggcgactgcttcatcctggacctgggcaacaacatccaccagtggtgtggttccaacagcaatcggtatgaaagactgaaggccacacaggtgtccaagggcatccgggacaacgagcggagtggccgggcccgagtgcacgtgtctgaggagggcactgagcccgaggcgatgctccaggtgctgggccccaagccggctctgcctgcaggtaccgaggacaccgccaaggaggatgcggccaaccgcaagctggccaagctctacaaggtctccaatggtgcagggaccatgtccgtctccctcgtggctgatgagaaccccttcgcccagggggccctgaagtcagaggactgcttcatcctggaccacggcaaagatgggaaaatctttgtctggaaaggcaagcaggcaaacacggaggagaggaaggctgccctcaaaacagcctctgacttcatcaccaagatggactaccccaagcagactcaggtctcggtccttcctgagggcggtgagaccccactgttcaagcagttcttcaagaactggcgggacccagaccagacagatggcctgggcttgtcctacctttccagccatatcgccaacgtggagcgggtgcccttcgacgccgccaccctgcacacctccactgccatggccgcccagcacggcatggatgacgatggcacaggccagaaacagatctggagaatcgaaggttccaacaaggtgcccgtggaccctgccacatatggacagttctatggaggcgacagctacatcattctgtacaactaccgccatggtggccgccaggggcagataatctataactggcagggtgcccagtctacccaggatgaggtcgctgcatctgccatcctgactgctcagctggatgaggagctgggaggtacccctgtccagagccgtgtggtccaaggcaaggagcccgcccacctcatgagcctgtttggtgggaagcccatgatcatctacaagggcggcacctcccgcgagggcgggcagacagcccctgccagcacccgcctcttccaggtccgcgccaacagcgctggagccacccgggctgttgaggtattgcctaaggctggtgcactgaactccaacgatgcctttgttctgaaaaccccctcagccgcctacctgtgggtgggtacaggagccagcgaggcagagaagacgggggcccaggagctgctcagggtgctgcgggcccaacctgtgcaggtggcagaaggcagcgagccagatggcttctgggaggccctgggcgggaaggctgcctaccgcacatccccacggctgaaggacaagaagatggatgcccatcctcctcgcctctttgcctgctccaacaagattggacgttttgtgatcgaagaggttcctggtgagctcatgcaggaagacctggcaacggatgacgtcatgcttctggacacctgggaccaggtctttgtctgggttggaaaggattctcaagaagaagaaaagacagaagccttgacttctgctaagcggtacatcgagacggacccagccaatcgggatcggcggacgcccatcaccgtggtgaagcaaggctttgagcctccctcctttgtgggctggttccttggctgggatgatgattactggtctgtggaccccttggacagggccatggctgagctggctgcc

SEQ ID NO: 10 - protein, 8 aa, synthetic construct
  REGION 1..8: note = A2D10 HCDR1
GYTFTEYT

SEQ ID NO: 11 - protein, 8 aa, synthetic construct
  REGION 1..8: note = A2D10 HCDR2
IYPHNGGT

SEQ ID NO: 12 - protein, 8 aa, synthetic construct
  REGION 1..8: note = A2D10 HCDR3
TEDLTFDY

SEQ ID NO: 13 - protein, 115 aa, synthetic construct
  REGION 1..115: note = A2D10
EVQLQQSGPELVKPGASVKISCKTSGYTFTEYTMHWVKQSHGKSLEWIGGIYPHNGGTNYNQKFKGKATLTVDKSSSTAYMELRSLTSEDSAVYYCTEDLTFDYWGQGTTLTVSS

SEQ ID NO: 14 - protein, 345 aa, synthetic construct
  REGION 1..345: note = A2D10
GAGGTCCAGCTGCAACAGTCTGGACCTGAGCTGGTGAAGCCTGGGGCTTCAGTGAAGATATCCTGCAAGACTTCTGGATACACATTCACTGAATACACCATGCACTGGGTGAAGCAGAGCCATGGAAAGAGCCTTGAGTGGATTGGAGGTATTTATCCTCACAATGGTGGTACTAACTACAACCAGAAGTTCAAGGGCAAGGCCACATTGACTGTAGACAAGTCCTCCAGCACAGCCTACATGGAGCTCCGCAGCCTGACATCTGAGGATTCTGCAGTCTATTACTGTACAGAAGATCTAACTTTTGACTACTGGGGCCAAGGCACCACTCTCACAGTCTCCTCA

SEQ ID NO: 15 - protein, 6 aa, synthetic construct
  REGION 1..6: note = A2D10 LCDR1
QDISNY

SEQ ID NO: 16 - skipped

SEQ ID NO: 17 - protein, 9 aa, synthetic construct
  REGION 1..9: note = A2D10 LCDR3
LQYSKLPFT

SEQ ID NO: 18 - protein, 107 aa, synthetic construct
  REGION 1..107: note = A2D10
DIQMTQTTSSLSASLGDRVTISCSASQDISNYLNWYQQKPDGTVKLLIYYTSSLHSGVPSRFSGSGSGTDYSLTISNLEPEDIATYHCLQYSKLPFTFGSGTKLEIK

SEQ ID NO: 19 - protein, 321 aa, synthetic construct
  REGION 1..321: note = A2D10
GATATCCAGATGACACAGACTACATCCTCCCTGTCTGCCTCTCTGGGAGACAGAGTCACCATCAGTTGCAGTGCAAGTCAGGACATTAGCAATTATTTAAACTGGTATCAGCAGAAACCAGATGGAACTGTTAAACTCCTGATCTATTACACATCAAGTTTACACTCAGGAGTCCCATCAAGGTTCAGTGGCAGTGGGTCTGGGACAGATTATTCTCTCACCATCAGCAACCTGGAACCTGAAGATATTGCCACTTACCATTGTCTACAGTATAGTAAGCTTCCATTCACGTTCGGCTCGGGGACAAAGTTGGAAATAAAA

SEQ ID NO: 20 - protein, 8 aa, synthetic construct
  REGION 1..8: note = HCDR1
GYTFSSYW

SEQ ID NO: 21 - protein, 8 aa, synthetic construct
  REGION 1..8: note = HCDR2
ILPGSGTT

SEQ ID NO: 22 - protein, 12 aa, synthetic construct
  REGION 1..12: note = HCDR3
ARSYDGYYVFDY

SEQ ID NO: 23 - protein, 119 aa, synthetic construct
  REGION 1..119: note = VH
QVQLKESGAELMKPGASVKISCKATGYTFSSYWIEWVKQRPGHGLEWIGEILPGSGTTNYNDKFKGKATFTADTSSNTAYMQLSNLTSEDSAVYYCARSYDGYYVFDYWGQGTTLTVSS

SEQ ID NO: 24 - protein, 357 aa, synthetic construct
  REGION 1..357: note = nucleotides encoding VH
CAGGTGCAGCTGAAGGAGTCAGGAGCTGAGCTGATGAAGCCTGGGGCCTCAGTGAAGATATCCTGCAAGGCTACTGGCTACACATTCAGTAGCTACTGGATAGAGTGGGTAAAGCAGAGGCCTGGACATGGCCTTGAGTGGATTGGAGAGATTTTACCTGGAAGTGGTACTACTAACTACAATGACAAGTTCAAGGGCAAGGCCACATTCACTGCAGATACATCCTCCAACACAGCCTACATGCAACTCAGCAACCTGACATCTGAGGACTCTGCCGTCTATTACTGTGCAAGATCCTATGATGGTTACTACGTCTTTGACTACTGGGGCCAAGGCACCACTCTCACAGTCTCCTCA

SEQ ID NO: 25 - protein, 10 aa, synthetic construct
  REGION 1..10: note = LCDR1
QSVDYDGDSY

SEQ ID NO: 26 - skipped

SEQ ID NO: 27 - protein, 9 aa, synthetic construct
  REGION 1..9: note = LCDR3
QQSNEDPRT

SEQ ID NO: 28 - protein, 111 aa, synthetic construct
  REGION 1..111: note = VL
DIELTQSPASLAVSLGQRATISCKASQSVDYDGDSYMNWYQQKPGQPPKLLIYAASNLESGIPARFSGSGSGTDFTLNIHPVEEEDAATYYCQQSNEDPRTFGGGTKLEIK

SEQ ID NO: 29 - protein, 333 aa, synthetic construct
  REGION 1..333: note = nucleotides encoding VL
GACATTGAGCTCACCCAATCTCCAGCTTCTTTGGCTGTGTCTCTAGGGCAGAGGGCCACCATCTCCTGCAAGGCCAGCCAAAGTGTTGATTATGATGGTGATAGTTATATGAACTGGTACCAACAGAAACCAGGACAGCCACCCAAACTCCTCATCTATGCTGCATCCAATCTAGAATCTGGGATCCCAGCCAGGTTTAGTGGCAGTGGGTCTGGGACAGACTTCACCCTCAACATCCATCCTGTGGAGGAGGAGGATGCTGCAACCTATTACTGTCAGCAAAGTAATGAGGATCCTCGGACGTTCGGTGGAGGCACCAAGCTGGAAATCAAA

SEQ ID NO: 30 - protein, 17 aa, synthetic construct
  REGION 1..17: note = HCDR3
ARSGVITARGDYYAMDY

SEQ ID NO: 31 - protein, 124 aa, synthetic construct
  REGION 1..124: note = VH
EVQLQQSGAELMKPGASVKISCKATGYTFSSYWIEWVKQRPGHGLEWIGEILPGSGTTNYNEKFKGKATFTVDTSSNTAYMQLSSLTSEDSAVYYCARSGVITARGDYYAMDYWGQGTSVTVSS

SEQ ID NO: 32 - protein, 372 aa, synthetic construct
  REGION 1..372: note = nucleotides encoding VH
GAGGTCCAGCTGCAGCAGTCAGGAGCTGAGCTGATGAAGCCTGGGGCCTCAGTGAAGATATCCTGCAAGGCTACTGGCTACACATTCAGTAGCTACTGGATAGAGTGGGTAAAGCAGAGGCCTGGACATGGCCTTGAGTGGATTGGAGAAATTTTACCTGGAAGTGGTACTACTAACTACAATGAGAAGTTCAAGGGCAAGGCCACATTCACTGTAGATACATCCTCCAACACAGCCTACATGCAACTCAGCAGCCTGACATCTGAGGACTCTGCCGTCTATTATTGTGCAAGATCAGGAGTGATTACGGCGAGAGGGGATTACTATGCTATGGACTACTGGGGTCAAGGAACCTCAGTCACCGTCTCCTCA

SEQ ID NO: 33 - protein, 111 aa, synthetic construct
  REGION 1..111: note = VL
DIVMTQSPASLAVSLGQRATISCKASQSVDYDGDSYMNWYQQKPGQPPKLLIYAASNLDSGIPARFSGSGSGTDFTLNIHPVEEEDAATYYCQQSNEDPRTFGGGTKLEIK

SEQ ID NO: 34 - protein, 333 aa, synthetic construct
  REGION 1..333: note = nucleotides encoding VL
GACATTGTAATGACCCAATCTCCAGCTTCTTTGGCTGTGTCTCTAGGGCAGAGGGCCACCATATCCTGCAAGGCCAGCCAAAGTGTTGATTATGATGGTGATAGTTATATGAACTGGTACCAACAGAAACCAGGACAGCCACCCAAACTCCTCATCTATGCTGCATCCAATCTAGATTCTGGGATCCCAGCCAGGTTTAGTGGCAGTGGGTCTGGGACAGACTTCACCCTCAACATCCATCCTGTGGAGGAGGAGGATGCTGCAACCTATTACTGTCAGCAAAGTAATGAGGATCCTCGGACGTTCGGTGGAGGCACCAAGCTGGAAATCAAA

SEQ ID NO: 35 - protein, 8 aa, synthetic construct
  REGION 1..8: note = HCDR1
GYTFSNYW

SEQ ID NO: 36 - protein, 9 aa, synthetic construct
  REGION 1..9: note = HCDR2
ILPGSYYST

SEQ ID NO: 37 - protein, 17 aa, synthetic construct
  REGION 1..17: note = HCDR3
ARSGMITTRGDYFAMDY

SEQ ID NO: 38 - protein, 125 aa, synthetic construct
  REGION 1..125: note = VH
EVQLQQSGAELMKPGASVKISCKATGYTFSNYWIEWIKQRPGHGLEWIGEILPGSYYSTNYNEKFKGKATFTADTSSNTAYIQLSSLTSEDSAVYYCARSGMITTRGDYFAMDYWGQGTSVTVSS

SEQ ID NO: 39 - protein, 375 aa, synthetic construct
  REGION 1..375: note = nucleotide encoding VH
GAGGTCCAGCTGCAGCAGTCAGGAGCTGAGCTGATGAAGCCTGGGGCCTCAGTGAAGATATCCTGCAAGGCTACTGGCTACACATTCAGTAACTACTGGATAGAGTGGATAAAGCAGAGGCCTGGACATGGCCTTGAATGGATTGGAGAGATTTTACCTGGAAGTTATTATAGTACTAACTACAATGAGAAGTTCAAGGGCAAGGCCACATTCACTGCAGATACTTCCTCCAACACAGCCTACATACAACTCAGCAGCCTGACATCTGAGGACTCTGCCGTCTATTACTGTGCAAGATCAGGAATGATTACGACGAGAGGGGATTACTTTGCTATGGACTACTGGGGTCAAGGAACCTCAGTCACCGTCTCCTCA

SEQ ID NO: 40 - protein, 111 aa, synthetic construct
  REGION 1..111: note = VL
DIVLTQSPASLAVSLGQRATISCKASQSVDYDGDSYMNWYQQKPGQPPKLLIYAASNLESGIPARFSGSGSGTDFTLNIHPVEEEDAATYYCQQSNEDPRTFGGGTKLEIK

SEQ ID NO: 41 - protein, 333 aa, synthetic construct
  REGION 1..333: note = nucleotide encoding VL
GACATTGTGCTCACCCAGTCTCCAGCTTCTTTGGCTGTGTCTCTAGGGCAGAGGGCCACCATCTCCTGCAAGGCCAGCCAAAGTGTTGATTATGATGGTGATAGTTATATGAACTGGTACCAACAGAAACCAGGACAGCCACCCAAACTCCTCATCTATGCTGCATCCAATCTAGAATCTGGGATCCCAGCCAGGTTTAGTGGCAGTGGGTCTGGGACAGACTTCACCCTCAACATCCATCCTGTGGAGGAGGAGGATGCTGCAACCTATTACTGTCAGCAAAGTAATGAGGATCCTCGGACGTTCGGTGGAGGCACCAAGCTGGAAATCAAA

SEQ ID NO: 42 - protein, 8 aa, synthetic construct
  REGION 1..8: note = HCDR2
ILPGSGST

SEQ ID NO: 43 - protein, 15 aa, synthetic construct
  REGION 1..15: note = HCDR3
ARTDDGYLSYFAMDY

SEQ ID NO: 44 - protein, 122 aa, synthetic construct
  REGION 1..122: note = VH
QVQLQQSGAELMKPGASVKISCKATGYTFSSYWIEWVKQRPGHGLEWIGEILPGSGSTNYNEKFKGKATFTADTSSNTAYMQLNSLTSEDSAVYYCARTDDGYLSYFAMDYWGQGTSVTVSS

SEQ ID NO: 45 - protein, 366 aa, synthetic construct
  REGION 1..366: note = nucleotide encoding VL
CAGGTTCAGCTGCAGCAGTCTGGAGCTGAGCTGATGAAGCCTGGGGCCTCAGTGAAGATATCCTGCAAGGCTACTGGCTACACATTCAGTAGCTACTGGATAGAGTGGGTTAAGCAGAGGCCTGGACATGGCCTTGAGTGGATTGGGGAGATTTTACCTGGAAGTGGTAGTACTAACTACAATGAAAAGTTCAAGGGCAAGGCCACATTCACTGCAGATACATCCTCCAACACAGCCTACATGCAACTCAACAGCCTGACATCTGAGGACTCTGCCGTCTATTACTGTGCGAGAACCGATGATGGTTACCTATCTTACTTTGCTATGGACTACTGGGGTCAAGGAACCTCAGTCACCGTCTCCTCA

SEQ ID NO: 46 - protein, 111 aa, synthetic construct
  REGION 1..111: note = VL
DILMTQTPASLAVSLGQRATISCKASQSVDYDGDSYMNWYQQKPGQPPKLLIYAASNLESGIPARFSGSGSGTDFTLNIHPVEEEDAATYYCQQSNEDPRTFGGGTKLEIK

SEQ ID NO: 47 - protein, 333 aa, synthetic construct
  REGION 1..333: note = nucleotide encoding VL
GACATTTTGATGACCCAGACTCCAGCTTCTTTGGCTGTGTCTCTAGGGCAGAGGGCCACCATCTCCTGCAAGGCCAGCCAAAGTGTTGATTATGATGGTGATAGTTATATGAACTGGTACCAACAGAAACCAGGACAGCCACCCAAACTCCTCATCTATGCTGCATCCAATCTAGAATCTGGGATCCCAGCCAGGTTTAGTGGCAGTGGGTCTGGGACAGACTTCACCCTCAACATCCATCCTGTGGAGGAGGAGGATGCTGCAACCTATTACTGTCAGCAAAGTAATGAGGATCCTCGGACGTTCGGTGGCGGCACCAAGCTGGAAATCAAA

SEQ ID NO: 48 - protein, 8 aa, synthetic construct
  REGION 1..8: note = HCDR2
ILPGGYNT

SEQ ID NO: 49 - protein, 17 aa, synthetic construct
  REGION 1..17: note = HCDR3
ARSGMITTTGDYYAMDY

SEQ ID NO: 50 - protein, 124 aa, synthetic construct
  REGION 1..124: note = VH
QVQLQQSGAEVMKPGASVKISCKATGYTFSSYWIEWIKQRPGHGLEWIGEILPGGYNTNSNENFKGKATFTADTSSNTAYMQLSSLTSEDSAVYYCARSGMITTTGDYYAMDYWGQGTSVTVSS

SEQ ID NO: 51 - protein, 372 aa, synthetic construct
  REGION 1..372: note = nucleotide encoding VH
CAGGTGCAGCTGCAGCAGTCTGGAGCTGAGGTGATGAAGCCAGGGGCCTCAGTGAAGATATCCTGCAAGGCTACTGGCTACACATTCAGTAGCTACTGGATAGAGTGGATAAAGCAGAGGCCTGGACATGGCCTTGAGTGGATTGGAGAGATTTTACCTGGAGGCTATAATACTAACTCCAATGAGAACTTCAAGGGCAAGGCCACATTCACTGCAGATACATCCTCCAACACAGCCTACATGCAACTCAGCAGCCTGACATCTGAGGACTCTGCCGTCTATTACTGTGCAAGATCAGGAATGATTACGACGACAGGGGATTACTATGCTATGGACTACTGGGGTCAAGGAACCTCAGTCACCGTCTCCTCA

SEQ ID NO: 52 - protein, 10 aa, synthetic construct
  REGION 1..10: note = LCDR1
QSVDYDGESY

SEQ ID NO: 53 - protein, 9 aa, synthetic construct
  REGION 1..9: note = LCDR3
QQSNDDPRT

SEQ ID NO: 54 - protein, 111 aa, synthetic construct
  REGION 1..111: note = VL
DIELTQSPASLAVSLGQRATISCKASQSVDYDGESYMNWYQQKPGQPPKLLIYAASNLESGIPARFSGSGSGTDFTLNIHPVEEEDAATYYCQQSNDDPRTFGGGTKLEIK

SEQ ID NO: 55 - protein, 333 aa, synthetic construct
  REGION 1..333: note = nucleotide encoding VL
GACATTGAGCTGACCCAATCTCCAGCTTCTTTGGCTGTGTCTCTAGGCCAGAGGGCCACCATCTCCTGCAAGGCCAGCCAAAGTGTTGATTATGATGGTGAGAGTTATATGAACTGGTACCAACAGAAACCAGGACAGCCACCCAAACTCCTCATCTATGCTGCATCCAATTTAGAGTCTGGGATCCCAGCCAGGTTTAGTGGCAGTGGGTCTGGGACAGACTTCACCCTCAACATCCATCCTGTGGAGGAGGAGGATGCTGCAACCTATTACTGTCAGCAAAGTAATGACGATCCTCGGACGTTCGGTGGAGGCACCAAGCTGGAAATCAAA

SEQ ID NO: 56 - protein, 8 aa, synthetic construct
  REGION 1..8: note = HCDR1
GYTFSRYW

SEQ ID NO: 57 - protein, 17 aa, synthetic construct
  REGION 1..17: note = HCDR3
ARSGVITTRGDYFAMDY

SEQ ID NO: 58 - protein, 125 aa, synthetic construct
  REGION 1..125: note = VH
QVQLQQSGAELMKPGASVKISCKATGYTFSRYWIEWIKQRPGHGLEWIGEILPGSYYSTNSNEKFKGKATFTADTSSNTAYMQLSSLTSEDSAVYYCARSGVITTRGDYFAMDYWGHGTSVTVSS

SEQ ID NO: 59 - protein, 375 aa, synthetic construct
  REGION 1..375: note = nucleotide encoding VL
CAGGTTCAACTGCAGCAGTCTGGAGCTGAGCTGATGAAGCCTGGGGCCTCAGTGAAGATATCCTGCAAGGCTACTGGCTACACATTCAGTAGGTACTGGATAGAGTGGATAAAGCAGAGGCCTGGACATGGCCTTGAGTGGATTGGAGAGATTTTACCTGGAAGTTATTATAGTACTAACTCCAATGAGAAGTTCAAGGGCAAGGCCACATTCACTGCAGATACATCCTCCAACACAGCCTACATGCAACTCAGCAGCCTGACATCTGAGGACTCTGCCGTCTACTACTGTGCAAGATCAGGAGTAATTACGACGAGAGGGGATTACTTTGCTATGGACTACTGGGGTCACGGAACCTCAGTCACCGTCTCCTCA

SEQ ID NO: 60 - protein, 111 aa, synthetic construct
  REGION 1..111: note = VL
DIVLTQSPASLAVSLGQRATISCKASQSVDYDGDSYMNWYQQKPGQPPKLLMYAASNLESGIPARFSGSGSGTDFTLNIHPVEEEDAATYYCQQSNEDPRTFGGGTKLEIK

SEQ ID NO: 61 - protein, 333 aa, synthetic construct
  REGION 1..333: note = nucleotide encoding VL
GACATTGTGCTCACCCAGTCTCCAGCTTCTTTGGCTGTGTCTCTAGGGCAGAGGGCCACCATCTCCTGCAAGGCCAGCCAAAGTGTTGATTATGATGGTGATAGTTATATGAACTGGTACCAACAGAAACCAGGACAGCCACCCAAACTCCTCATGTATGCTGCATCCAATCTAGAATCTGGGATCCCAGCCAGGTTTAGTGGCAGTGGGTCTGGGACAGACTTCACCCTCAACATCCATCCTGTGGAGGAGGAGGATGCTGCTACCTATTACTGTCAGCAAAGTAATGAGGATCCTCGGACGTTCGGTGGAGGCACCAAGCTGGAAATCAAA

SEQ ID NO: 62 - protein, 17 aa, synthetic construct
  REGION 1..17: note = HCDR3
ARSGIITTRGDYFAMDY

SEQ ID NO: 63 - protein, 125 aa, synthetic construct
  REGION 1..125: note = VH
QVQLQQSGAELMKPGASVKISCKATGYTFSNYWIEWIKQRPGHGLEWIGEILPGSYYSTNYNEKFKDKATFTADTSSNTAYIQLSSLTSEDSAVYYCARSGIITTRGDYFAMDYWGQGTSVTVSS

SEQ ID NO: 64 - protein, 375 aa, synthetic construct
  REGION 1..375: note = nucleotide encoding VH
CAGGTTCAGCTGCAGCAGTCTGGAGCTGAGCTGATGAAGCCTGGGGCCTCAGTGAAGATATCCTGCAAGGCTACTGGCTACACATTCAGTAACTACTGGATAGAGTGGATAAAGCAGAGGCCTGGACATGGCCTTGAGTGGATTGGAGAGATTTTACCTGGAAGTTATTATAGTACTAACTACAATGAGAAGTTCAAGGACAAGGCCACATTCACTGCAGATACATCCTCCAACACAGCCTACATACAACTCAGCAGCCTGACATCTGAGGACTCTGCCGTCTATTATTGTGCAAGATCAGGAATAATTACGACGAGAGGGGATTACTTTGCTATGGACTACTGGGGTCAAGGAACCTCAGTCACTGTCTCCTCA

SEQ ID NO: 65 - protein, 124 aa, synthetic construct
  REGION 1..124: note = VH
QVQLQQSGAELMKPGASVKISCKATGYTFSNYWIEWVKQRPGHGLEWIGEILPGSGSTNYNEKFKGKATFTADTSSNTAYMQLSSLTSEDSAVYYCARSGMITTRGDYFAMDYWGQGTSVTVSS

SEQ ID NO: 66 - protein, 372 aa, synthetic construct
  REGION 1..372: note = nucleotide encoding VH
CAGGTGCAGCTGCAGCAGTCTGGAGCTGAGCTGATGAAGCCTGGGGCCTCAGTGAAGATATCCTGCAAGGCTACTGGCTACACATTCAGTAACTACTGGATAGAGTGGGTAAAGCAGAGGCCTGGACATGGCCTTGAGTGGATTGGAGAGATTTTACCTGGAAGTGGTAGTACTAACTACAATGAGAAGTTCAAGGGCAAGGCCACATTCACTGCAGATACATCCTCCAACACAGCCTACATGCAACTCAGCAGCCTGACATCTGAGGACTCTGCCGTCTATTACTGTGCAAGATCGGGGATGATTACGACGAGAGGGGATTACTTTGCTATGGACTACTGGGGTCAAGGAACCTCAGTCACCGTCTCCTCA

SEQ ID NO: 67 - protein, 9 aa, synthetic construct
  REGION 1..9: note = LCDR3
QQSYDDPRA

SEQ ID NO: 68 - protein, 111 aa, synthetic construct
  REGION 1..111: note = VL
DIELTQSPASLAVSLGQRATISCKASQSVDYDGESYMNWYQQKPGQPPKLLIYAASNLESGIPARFSGSGSGTDFTLNIHPVEEEDAATYYCQQSYDDPRAFGGGTKLEIK

SEQ ID NO: 69 - protein, 333 aa, synthetic construct
  REGION 1..333: note = nucleotide encoding VL
GACATTGAGCTGACCCAATCTCCAGCTTCTTTGGCTGTGTCTCTAGGCCAGAGGGCCACCATCTCCTGCAAGGCCAGCCAAAGTGTTGATTATGATGGTGAGAGTTATATGAACTGGTACCAACAGAAACCAGGACAGCCACCCAAACTCCTCATCTATGCTGCATCCAATCTAGAATCTGGGATCCCAGCCAGGTTTAGTGGCAGTGGGTCTGGGACAGACTTCACCCTCAACATCCATCCTGTGGAGGAGGAGGATGCTGCAACCTATTACTGTCAGCAAAGTTATGACGATCCTCGGGCGTTCGGTGGAGGCACCAAGCTGGAAATCAAA

SEQ ID NO: 70 - protein, 8 aa, synthetic construct
  REGION 1..8: note = HCDR1
  SITE 5: note = misc_feature - Xaa = Ser Thr
  SITE 6: note = misc_feature - Xaa = Glu Asn Arg Ser
  SITE 8: note = misc_feature - Xaa = Thr Trp
  source 1..8: note = HCDR1 general formula
GYTFXXYX

SEQ ID NO: 71-75 - skipped (5 entries)

SEQ ID NO: 76 - DNA, 35 bp, synthetic construct
  misc_feature 1..35: note = pCMV-flag-DIRFlag-DIR
  source 1..35: mol_type = other DNA
ccatggaggcccgaattcggatggttgcaactggc

SEQ ID NO: 77 - DNA, 44 bp, synthetic construct
  misc_feature 1..44: note = pCMV-flag-DIRFlag-DIR
  source 1..44: mol_type = other DNA
actcatcaatgtatcttatcttatggagagaagatgttagaaaa

SEQ ID NO: 78 - DNA, 30 bp, synthetic construct
  misc_feature 1..30: note = pcDNA3.1-DDIT4L-myc-his
  source 1..30: mol_type = other DNA
gccaccatggttgcaactggcagtttgagc

SEQ ID NO: 79 - DNA, 30 bp, synthetic construct
  misc_feature 1..30: note = pcDNA3.1-DDIT4L-myc-his
  source 1..30: mol_type = other DNA
gaattccaccacactggactagtggatccg

SEQ ID NO: 80 - DNA, 32 bp, synthetic construct
  misc_feature 1..32: note = Gelsolin-pEGFP
  source 1..32: mol_type = other DNA
tcaagcttcgaattcatggctccgcaccgccc

SEQ ID NO: 81 - DNA, 35 bp, synthetic construct
  misc_feature 1..35: note = Gelsolin-pEGFP
  source 1..35: mol_type = other DNA
cgggcccgcggtaccggcagccagctcagccatgg

SEQ ID NO: 82 - DNA, 32 bp, synthetic construct
  misc_feature 1..32: note = pcDNA3.1-Gelsolin-myc-his
  source 1..32: mol_type = other DNA
gtggaattcgccaccatggctccgcaccgccc

SEQ ID NO: 83 - DNA, 35 bp, synthetic construct
  misc_feature 1..35: note = pcDNA3.1-Gelsolin-myc-his
  source 1..35: mol_type = other DNA
ccctctagactcgagggcagccagctcagccatgg

SEQ ID NO: 84 - RNA, 19 nt, synthetic construct
  misc_feature 1..19: note = DIR siRNA1
  source 1..19: mol_type = other RNA
tttggaaaggagtctcctc

SEQ ID NO: 85 - RNA, 19 nt, synthetic construct
  misc_feature 1..19: note = DIR siRNA1
  source 1..19: mol_type = other RNA
gaggagactcctttccaaa

SEQ ID NO: 86 - RNA, 19 nt, synthetic construct
  misc_feature 1..19: note = DIR siRNA2
  source 1..19: mol_type = other RNA
tgttagaaaatttggaaag

SEQ ID NO: 87 - RNA, 19 nt, synthetic construct
  misc_feature 1..19: note = DIR siRNA2
  source 1..19: mol_type = other RNA
ctttccaaattttctaaca

SEQ ID NO: 88 - DNA, 23 bp, synthetic construct
  source 1..23: mol_type = other DNA
  misc_feature 1..23: note = Knock in QDLIR sgRNA
atttcagagttgttggacggtgg

SEQ ID NO: 89 - DNA, 3000 bp, synthetic construct
  misc_feature 1..3000: note = 5
  source 1..3000: mol_type = other DNA
caacttgactatatttggaatgaactacaatccagaattggaaggctcaccagtgacccttatctggaggcttggagatccttatctggatcttggtatggagatcttgagccatagtgactatggattccagaagattgaatctcagagtttaaggaacacacctttaacctgggctacacctttcatctgggattaaaggtgtggtggaacacacctttaatctgggctacaccttctgctggagacaatataaggacattggaagaagggagtctagctcttgctccttcgcctgcttgctgcgtgagactgagtaactgctagatccttggacttccattcacagcttctactgaacaattgttgggaattgggctgccgactgtaagtcatcaataaattcctttactatccataagttctgtgactctagagaaccctgactaatacagtagtcttggtttttcttgattctgtttgaatccttaaaatatttcattttcttaagtcatctacttagatgcaaagatagaagttggtgagagcatgtggcttgaaatcatgttaggtgacctttaagaaagacaatctctgtcggttactgcaggtatatgctctacacctcctgattcctcctgccctaagcttcctgatagcatcactcgttcagtcaaaaagaatgctcttatttgaaatttttgcatatgggtaaattgccttctgagataaaagcccagagagtgatataaaattgtagctaggtgagccaaaagtaaataccacattctagaactttctataactttgtcccggtggaagtatgaattatgcctaaatacccgagtggaaatgctgcattttctctattctacccacgtccattctgatcacttactatcataacactaataacattccttgaagcagggaggacgcagctgtcattaacaaggctgactagataaggaccagcggctctgtagcagctaaaggacccattctaaccggcttaaatgggattgcttgttttccacttttgttattaaaatagaagtggaaatctgctttccccagcctatcagcatcccgtgcctgagcctgcctgaccttgagcagtgcagctgcttcgggagagttaaaaatggaccttcaagctggctttagtttctgttgctctgcctgcaagtgtcctcccactgatctgtttatcacactctctttaccacttttgttgttgtttttccttctgagagtttttttagcctggacagcggatcctacttctcaaggccctaacctgcaggtccttccttgcacgtggggacccaaagtgtgcgggagtggtgctggaacctggccttgaatgaggttcaccctcaccccaagtatctcggtctcttccttttctgatccacctcaaccatctcagcaacctcagcaacctcgctgggaacgcccacccattgcaaaccctgtgccactggcgcagggcagcaggaagggtggcttagtaaagttagaagaaaacgtttggcatcgtgcttttagtggtgtcccagaccctctgttccctcttgctcaagactccccggaaagagtcgcagagcttatcctagcaggacaactctttattctcatgccccacaagctttttaaagaccactaaagcttaaacttcttcccaaacaagcccaccgggaacttttgcttctgggaatggcaattgctcctaactatcctgcggctggagcaggcaactgagatcctgttagtggttttgtttagtttcttggcactggccctcttcaattcaagttctgtgcctttcgaagccaggtcttagaacagggccaggctcgccctggccgcggagaaaaacggtttagtcacagatgtagtatccccaaagatgccccattgattcctgagtgcagctgaagctagagagcccttaccacatcccgaccacctgcggggagactgggtgcggactggagctgatgggttagagtcagaacatgggcataaaggatgctcacagagcacagtgtcaactaagccaaatacttattcagaatgacacagcaaagttttgggtcatgcctaacaggacctggagcttctagctgcttgaaaagttccatagccaaaacctgagcagtctgagcctggaagcaggcaagctgtgggcaggggctcacgccaaagaatctaggttagtggccgaagggagatgctctttaggagggtgaccagtggccaactcagggtgaccagtggccaactcaggaagcagcaggtgtccgcccaaggcgaggctgatcaccaactcccaggggcttgcctgggcccctgcctgggaaggaactgaaaggtgacctgaccctgcaggggcgggccggggcacgggcccgagcgagtggcgcaggtgggcgtgccggccaggaggagaggcgggacctataaagcgctctccattcgggaggcggagcggccgggtgcagcctgtgctggtgggcgcggtggcccgcagccttcggcttgctgcaggactgtgcaggggaccactgtccaagcttcggactactgaggggcgcctgcctcggtttacccttcagcgtctggtgaaatccggcaggtgagcgacccgaggaggcgggatagggcagggtcgcttcccagttgtgctgactttccagctacttccagcctgttggctttagttggcgcctccgctcctagggctttgtcaacttgagttgctaaggctggtccctccctttggaagggcagtgcccgggctagttcgccctggcgatgccgggactctgaggagcctgtgcacttcttgcgtgcttttgcaaacttctcactttttcctcccagcgcctagggaaagatccgttctgctccgcgagggaaacagagccgttgaccatggttgcaacgggcagtttgagcagtaagaacccggccagcatttcagagttgttggac

SEQ ID NO: 90 - DNA, 195 bp, synthetic construct
  misc_feature 1..195: note = QDLIR 64
  source 1..195: mol_type = other DNA
tgtggctatcacccagagagcctgctaagtggtgagtgtccccgctgtccacccttctcccctcccaaggtcggtgcctctggatctattgggtgggcgggctttcgacttcctcccctacctctatgtaggaggtgccacaaaatccatctgaggagactcctttccaaattttctaacatcttctctccatga

SEQ ID NO: 91 - DNA, 3000 bp, synthetic construct
  misc_feature 1..3000: note = 3
  source 1..3000: mol_type = other DNA
ggtggctatcaccctgggagtctgctaagtggtgagtctctgggctgtccacctctttcctatccgaaggttgcggggcccctctctagtgtaagcgtccctgcctgagtgcgcgagacttcatctcctcctagagacacagaggactatgaaacccatctgagatctctttctaaacttcctttgcattgtctgcccaccaaaaacaaacgtaaggggaataatgcgttgttccagtctgctaagaggctcttggggatgaagttccctatctcatggttggaacattaagtgtacaggctgggtgtgtttaaagacatgcgcttacttgtgtagctagcaccaccacgtccgtcccccctccccccccccccccaaattctcccttttctgtttgccacctaatccttctctttcccgtctccagaagaccatccttcggcattttgttaccacgttagttttgcttttagaatgttaaataataagtgtatatgctcttctcagttcggtttgctttcccaccgtgtgatgttgtagagttatacacttacctcatcagtgagttccttttcgttgctaagtaagattctattatgaaatgcacccactgtgcattaatgtcagaagaaaacttgaacagccctggttctacaggaatcatcatttgcaacttgaaacgtcaatttctaatctgacagactattcaactatggaagagtggtgtgagcatatattaagtggcttaagctctttagattttcttcatctataagataatattataattctaaatttgtctgtcttcaatgtggataaaaatacagatatgatttggaatctatttgttggaatttaaaaaataaaacaaaaaacaaaaaacaagcagtgccctctaagtgagctaatgacatagaaaaccaggagaggagaggaaggctcgtggccgcagtgtggcatggcacccggccaagtagtaggattaatttggaaggtaggtgaccaaatgcagagctatcttttttcctctgagtaaacctaactttgttttcctgggactgttttgttttgctcagctaagaaaaactgacccagcccggttataaataaactcaggaacctcaaaagtcctctctcctctgcgagcaaacttgaatcaaacaggtcaaagccaacactggacctccaggccatcctagtaaggacttctaacgaaaactaaggctggtagatcattagcattgggacaggctcactttacagcgtttgaaaccattctgcacgccaacggtccctttgttaagcaatagtgatgatttttattccagatgttctgcatggacttgtgaaaaaaaactaaaataaacttggaaaaccctacagagagagcaagggggaaaggagatcactagtaatcttggatgaccttggacagatttttgccacataatcctcaagactacggggagagaagaaattgtaaaagagggttgttttaacctattcattatgtttatcagagtctttagggcatagatgagctttcagtcctgaaaggttagaaggcctgttctattacctacatggttaacagcaaaattgagatgagagaaagcagtattaaaagcaggtagatatgaagctagaagtggccagtcttactatgccagtaagacctcgtacaccttgcttctctgttcactaaaactttcatttctttcagatttcgactactgggattatgttgtccctgagcccaacctcaacgaggtggtatttgaagagacaacatgccagaatttggttaaaatgttggagaactgtctgtccagatcaaagcaaaccaaacttggttgctctaaggtcttggtccctgagaaactgacccagagaattgctcaagatgtcctgcggctctcgtccacggagccctgcggccttcggggttgtgttatgcacgtgaacttggagattgaaaatgtatgtaaaaagctggataggatcgtgtgtgatgctagcgtggtgccgacctttgagctcacgcttgtgtttaagcaggagagctgcccgtggaccagcctcaaggacttcttctttagcagaggtcgcttctcctcaggccttaagcgaactctgattctcagctcaggatttcgacttgtgaagaaaaaactgtactccctgattggaacgacagtcattgaagagtgctaaggaggaaaaacaattaaaggcccctaatgagtggataataaacctctgaagctatccagccagtcatttgtagtttgcctgcttgccctcaccaggaaatcccagatttaggcccttttccttctgtgtgtctcacccatagcaacccactttaaaggctgattttttttttttttgtccagcttttaagacataattcaagagagcaaattgcccacatatgtgtccatatgggatagaatggaataaggaggaaaaagaagcaatctcctttaattttatatttggtctcatatttagcaggtagtcttagcaacagagcaagatccactttgcctaatttgactttcatgtgcccagggcttgctgttattgtacccgcctctctctctctctctctctctctctctgtgtgtgtgtgtgtgtgtgtgtgtatatatatatatctgtctgtctctctctgtctctctgtctctctctctctcctcccctccctccctctctgagagccatcttttcaatgacaggacctgacaagatgatgtgcagccccatcaaaacatatagagatctgcactaccagcttcctccctgaatttgaagagcttttacacaagagggtacagttaaattgatccgctggattaaaacatcaccttacatagagcgaataaacatcacagtgacaagagcatggcttccctgcctggtggtctccccacacccgtgcccaggagacacgagaagtgtgcctcttactgcaatgattacatgatggctttcagt

SEQ ID NO: 92 - DNA, 4599 bp, Homo sapiens
  source 1..4599: mol_type = genomic DNA
gctactgcgaggagccggcgcagggtggcccgggaggggtgagcagggtgccgctggctgctggggtctgcaggtcaccgagtccccaggagaggggactcctaagaagccacctgcctgtgtttacccggcagcgagcgcgcaggcccccgcgaactcctggcaggtgagcgaagctgcggccttggtgggggcagcggggccggggggcgctccgcggggcaggtcgcttccaagttttgcgaactgttgagttagtttcaggttgcggctccgctcccagggctttgtcaaattgagttgcagaggccggttccacccctttggcaaaggagttcctccgctagttcgctcccgggacgccgggcattttaggagcctctgcacgactcgcctgcttttgcaaatccgtctcttctcgcctcattttttccagcgctcaggaaaggccgttgcgcctcgcgaaggaaacagagccgttgaccatggttgcaactggcagtttgagcagcaagaacccggccagcatttcagaattgctggactgtggctatcacccagagagcctgctaagtggtgagtgtccccgctgtccacccttctcccctcccaaggtcggtgcctctggatctattgggtgggcgggctttcgacttcctcccctacctctatgtaggaggtgccacaaaatccatctgaggagactcctttccaaattttctaacatcttctctccatgatagaaacaaaagtagcaaaagtagaatacccgagggctgcatctttctagtctggtgccagtaggccccttgggattaagttccttatcttacatgattgtgaagaacacagttatgtgtgttttagcaaatgtatttaccctgtaatcaatatcgcccctccccctgaattccgacgcacctatttgccaggtattcctcactctcccctgactccagggaactactgatctgatttttatcattccaagttagttttgcctttaggtaagtggaaccatacagtaggtattcttttgtgtctggtttctttcccgcagcctaatgtttttgagattcttttatgtccgttgcttaaatcagtgtgttcgtgtttattgtttattactgagtaggattttcagtcgtggatatatccattattccatttttaatgtgagaaggaaactgttgaacagcagcggtgcttgacttgctgtcatttggaattttaacagcagtttctaggtgaacacactgctctgacactaaagagctgtaagagcatagataaactgcttaagctcttcgtgtttttctcctttcaaggtgaagtggttgatgacctaatttacaggccagaactccaaacttacacgaagtggagaggaaaagccagtggctgatgaaggtggagtaggcttagagagaggagctgggagggcatctgcctgcaccttgttcatttgactccgtgtggtgtggcatcctgccaaggggtaggattaatttgaggtgtaggtgaccaaatgcagagctatctcttttcctttgagcccagctaattttatttccctaggactattttgttttgcttggctaagaaaaaccacccagccggttacaaatatcctcatgaacctcaaaggtcttctctgcacaatttttaattaaagaggctaaagctaaaattgggacctacaggccactccagtaaagacttaaagacacaaatttgatagatctttaatataactcttaaagctttaatacaactcttcaaacataatagtaaaaattctttattttacaatacatgtattcctacagttagaaagtaacaaccccttagtccaaaaaacaaagttataactttttattccagaagtaatgcatgttttctgtaaaacaaaattagaaaacccccataagcaagtaggagaaaagaaaagaaaatcaccaataatctgggataatcacaagtagatttttgatgcatagtcttcacggttgtgtgtgtgttttgtgtacacacataaatttaaagaaaagtggttacatcctatctactctatttatctaaacctttatttcatacatgaactttcattcatgagagcttaaattattcgctatattacctagctagttaacagttaattgaggtcagctgactctgaaacaaatacaagaaaaaggcagacatggtagatagaggtaaccaatgttgatatcttggtgttttttttctactcttaaattttttcttctgtatctaaaaagaaaactccatttcttacagattttgactactgggattatgttgttcctgaacccaacctcaacgaggtaatatttgaggaatcaacttgccagaatttggttaaaatgctggagaactgtctgtccaaatcaaagcaaactaaacttggttgctcaaaggtccttgtccctgagaaactgacccagagaattgctcaagatgtcctgcggctttcctcaacggagccctgcggcttgcgaggttgtgttatgcacgtgaacttggaaattgaaaatgtatgtaaaaagctggataggattgtgtgtgattctagcgtcgtacctacttttgagcttacacttgtgtttaagcaggagaactgctcatggactagcttcagggactttttctttagtagaggtcgcttctcctctggtttcaggagaactctgatcctcagctcaggatttcgacttgttaagaaaaaactttactcactgattggaacaacagtgattgaagggtcctaaaaagggaaaatatataaagattatttcatgattgggtagtaaaactattcagctagtcagctaaagtcatttgtagtttgccccacctgccctaaataagaaaccccaaatgtagtctcttttctttctgtgtttcacattcatagcaactgcagctaacaggctgattttctggcctttggagaagtgattcaaaatagtgtagattttctgcatagatcccatttttgtacagaattgaatgggatggaataggtaagcaaaagtagaagcccatttgagttttacatttgattccacaatttggtttcaggtaggcttggtaatagactatataaaccagatttgcctattttgattttcatatggcttttttttctgtaagttttcagaggattttttaaatcacagaatcatactaaatgatatttagcctatcaaaacttccaaaagcccacaccaccagttcctgactcaaatttgaagggtttttagacaggagggtaggattaagtaggtgagtttaattaaagcttaaccctaggtaagagtaaatgagaaatattacggcaataatggaactgcttcactgtttcttggtgacttcctcactctaatgttttaaagaggcaacaaaagcttgtggtgccatttcagtaaccacggtgttgttttagatgcctttataagctcagtttcccctgttcttaagtgttgaatactgtctttaaactagaaaaatgcaaaatattgaactgatatttttgtgtgtagttgattactcttccattgagtgaatgatgaatacctgtgaggataggaaattagttctgagatctagtccctctctgattcacttagtaatctatcctcttttcagtattacatgtgcttaatctcagatgaaccatttcaccatggcagtgttatctcatctctgggcttttctgggaattgaagtatctctccttaaccccaattgtcaagggtagtagctgtatactaccactttgaattattgaaacgggtcaatttacgaagtctgcattggctatggagatatggtttatagtacagcctagagaatgaaactcaccgtccagataaccatgcatgcacccagattttttccaccttggatacctgtcactagggaataataaaggcctgattttttgtcttattccaactaagtagatcattatctctttccttttttatgttaatgagagaatttagcctccactcaacaatgttcaattcagcaaggctttcatatccttgctgtgggtcgtggataaggagcttattcaggtttcctgccctagctattagctccacttcacatgctggagaccggcgtagggacagatgtattcatcctggtgttactgaaaaacaggtgtgatcctgttactgatactataagtgacctaaaatgtcactgttcaaattagccagtgttctaacaaactaaactcttcaaatgcttggaaagatactacaaagccaatctttatagaattgggccaagataaatctatgttgttttgcatggctattgttaagctccaaaggttcactgtgtttctgccgctgtcctggagttgtcaccactgactgggcaaggcttcttgggcatggatgtagaactgttgtccttttcccactaacagttatctttgactctcttgcctgttatgcttacaaaatggtgatggcttatggaaggctgttaaattaatattcctgttaaaggaaattaaagtttgtctatttttgacaataaaacattatatatttttaa

SEQ ID NO: 93 - DNA, 4163 bp, Homo sapiens
  source 1..4163: mol_type = genomic DNA
cgctcaggaaaggccgttgcgcctcgcgaaggaaacagagccgttgaccatggttgcaactggcagtttgagcagcaagaacccggccagcatttcagaattgctggactgtggctatcacccagagagcctgctaagtggtgagtgtccccgctgtccacccttctcccctcccaaggtcggtgcctctggatctattgggtgggcgggctttcgacttcctcccctacctctatgtaggaggtgccacaaaatccatctgaggagactcctttccaaattttctaacatcttctctccatgatagaaacaaaagtagcaaaagtagaatacccgagggctgcatctttctagtctggtgccagtaggccccttgggattaagttccttatcttacatgattgtgaagaacacagttatgtgtgttttagcaaatgtatttaccctgtaatcaatatcgcccctccccctgaattccgacgcacctatttgccaggtattcctcactctcccctgactccagggaactactgatctgatttttatcattccaagttagttttgcctttaggtaagtggaaccatacagtaggtattcttttgtgtctggtttctttcccgcagcctaatgtttttgagattcttttatgtccgttgcttaaatcagtgtgttcgtgtttattgtttattactgagtaggattttcagtcgtggatatatccattattccatttttaatgtgagaaggaaactgttgaacagcagcggtgcttgacttgctgtcatttggaattttaacagcagtttctaggtgaacacactgctctgacactaaagagctgtaagagcatagataaactgcttaagctcttcgtgtttttctcctttcaaggtgaagtggttgatgacctaatttacaggccagaactccaaacttacacgaagtggagaggaaaagccagtggctgatgaaggtggagtaggcttagagagaggagctgggagggcatctgcctgcaccttgttcatttgactccgtgtggtgtggcatcctgccaaggggtaggattaatttgaggtgtaggtgaccaaatgcagagctatctcttttcctttgagcccagctaattttatttccctaggactattttgttttgcttggctaagaaaaaccacccagccggttacaaatatcctcatgaacctcaaaggtcttctctgcacaatttttaattaaagaggctaaagctaaaattgggacctacaggccactccagtaaagacttaaagacacaaatttgatagatctttaatataactcttaaagctttaatacaactcttcaaacataatagtaaaaattctttattttacaatacatgtattcctacagttagaaagtaacaaccccttagtccaaaaaacaaagttataactttttattccagaagtaatgcatgttttctgtaaaacaaaattagaaaacccccataagcaagtaggagaaaagaaaagaaaatcaccaataatctgggataatcacaagtagatttttgatgcatagtcttcacggttgtgtgtgtgttttgtgtacacacataaatttaaagaaaagtggttacatcctatctactctatttatctaaacctttatttcatacatgaactttcattcatgagagcttaaattattcgctatattacctagctagttaacagttaattgaggtcagctgactctgaaacaaatacaagaaaaaggcagacatggtagatagaggtaaccaatgttgatatcttggtgttttttttctactcttaaattttttcttctgtatctaaaaagaaaactccatttcttacagattttgactactgggattatgttgttcctgaacccaacctcaacgaggtaatatttgaggaatcaacttgccagaatttggttaaaatgctggagaactgtctgtccaaatcaaagcaaactaaacttggttgctcaaaggtccttgtccctgagaaactgacccagagaattgctcaagatgtcctgcggctttcctcaacggagccctgcggcttgcgaggttgtgttatgcacgtgaacttggaaattgaaaatgtatgtaaaaagctggataggattgtgtgtgattctagcgtcgtacctacttttgagcttacacttgtgtttaagcaggagaactgctcatggactagcttcagggactttttctttagtagaggtcgcttctcctctggtttcaggagaactctgatcctcagctcaggatttcgacttgttaagaaaaaactttactcactgattggaacaacagtgattgaagggtcctaaaaagggaaaatatataaagattatttcatgattgggtagtaaaactattcagctagtcagctaaagtcatttgtagtttgccccacctgccctaaataagaaaccccaaatgtagtctcttttctttctgtgtttcacattcatagcaactgcagctaacaggctgattttctggcctttggagaagtgattcaaaatagtgtagattttctgcatagatcccatttttgtacagaattgaatgggatggaataggtaagcaaaagtagaagcccatttgagttttacatttgattccacaatttggtttcaggtaggcttggtaatagactatataaaccagatttgcctattttgattttcatatggcttttttttctgtaagttttcagaggattttttaaatcacagaatcatactaaatgatatttagcctatcaaaacttccaaaagcccacaccaccagttcctgactcaaatttgaagggtttttagacaggagggtaggattaagtaggtgagtttaattaaagcttaaccctaggtaagagtaaatgagaaatattacggcaataatggaactgcttcactgtttcttggtgacttcctcactctaatgttttaaagaggcaacaaaagcttgtggtgccatttcagtaaccacggtgttgttttagatgcctttataagctcagtttcccctgttcttaagtgttgaatactgtctttaaactagaaaaatgcaaaatattgaactgatatttttgtgtgtagttgattactcttccattgagtgaatgatgaatacctgtgaggataggaaattagttctgagatctagtccctctctgattcacttagtaatctatcctcttttcagtattacatgtgcttaatctcagatgaaccatttcaccatggcagtgttatctcatctctgggcttttctgggaattgaagtatctctccttaaccccaattgtcaagggtagtagctgtatactaccactttgaattattgaaacgggtcaatttacgaagtctgcattggctatggagatatggtttatagtacagcctagagaatgaaactcaccgtccagataaccatgcatgcacccagattttttccaccttggatacctgtcactagggaataataaaggcctgattttttgtcttattccaactaagtagatcattatctctttccttttttatgttaatgagagaatttagcctccactcaacaatgttcaattcagcaaggctttcatatccttgctgtgggtcgtggataaggagcttattcaggtttcctgccctagctattagctccacttcacatgctggagaccggcgtagggacagatgtattcatcctggtgttactgaaaaacaggtgtgatcctgttactgatactataagtgacctaaaatgtcactgttcaaattagccagtgttctaacaaactaaactcttcaaatgcttggaaagatactacaaagccaatctttatagaattgggccaagataaatctatgttgttttgcatggctattgttaagctccaaaggttcactgtgtttctgccgctgtcctggagttgtcaccactgactgggcaaggcttcttgggcatggatgtagaactgttgtccttttcccactaacagttatctttgactctcttgcctgttatgcttacaaaatggtgatggcttatggaaggctgttaaattaatattcctgttaaaggaaattaaagtttgtctatttttgacaataaaacattatatatttttaa

SEQ ID NO: 94 - DNA, 582 bp, Homo sapiens
  source 1..582: mol_type = genomic DNA
atggttgcaactggcagtttgagcagcaagaacccggccagcatttcagaattgctggactgtggctatcacccagagagcctgctaagtgattttgactactgggattatgttgttcctgaacccaacctcaacgaggtaatatttgaggaatcaacttgccagaatttggttaaaatgctggagaactgtctgtccaaatcaaagcaaactaaacttggttgctcaaaggtccttgtccctgagaaactgacccagagaattgctcaagatgtcctgcggctttcctcaacggagccctgcggcttgcgaggttgtgttatgcacgtgaacttggaaattgaaaatgtatgtaaaaagctggataggattgtgtgtgattctagcgtcgtacctacttttgagcttacacttgtgtttaagcaggagaactgctcatggactagcttcagggactttttctttagtagaggtcgcttctcctctggtttcaggagaactctgatcctcagctcaggatttcgacttgttaagaaaaaactttactcactgattggaacaacagtgattgaagggtcctaa

SEQ ID NO: 95 - protein, 193 aa, Homo sapiens
MVATGSLSSKNPASISELLDCGYHPESLLSDFDYWDYVVPEPNLNEVIFEESTCQNLVKMLENCLSKSKQTKLGCSKVLVPEKLTQRIAQDVLRLSSTEPCGLRGCVMHVNLEIENVCKKLDRIVCDSSVVPTFELTLVFKQENCSWTSFRDFFFSRGRFSSGFRRTLILSSGFRLVKKKLYSLIGTTVIEGS